European Patent Application EP 4 174 090 A1, published May 3, 2023. Title: ANTI-CD133 SINGLE-CHAIN ANTIBODY AND USE THEREOF IN PREPARATION OF DRUG FOR TREATING TUMOR. Applicant: Beijing Neurosurgical Institute. The sequence listing filed with the application follows.

SEQUENCE LISTING (10 sequences)

SEQ ID NO: 1 - protein, 244 aa, Artificial Sequence
  This sequence is synthesized in lab.
QVQLVQSGAEVKKPGASVKVSCKASGYTFTDFEMHWVRQAPGQGLEWMGDIDPGTGDTAYNLKFKGRVTMTTDTSTSTAYMELRSLRSDDTAVYYCALGAFVYWGQGTLVTVSSGSTSGGGSGGGSGGGGSSDVVMTQSPLSLPVTPGEPASISCRSSQSLANSYGNTYLSWYLQKPGQSPQLLIYGISNRFSGVPDRFSGSGSGTDFTLKISRVEAEDVGVYYCLQGTHQPYTFGQGTKLEIK

SEQ ID NO: 2 - DNA, 732 bp, Artificial Sequence
  This sequence is synthesized in lab.
caggttcagctggtgcagtctggagctgaggtgaagaagcctggggcctcagtgaaggtctcctgcaaggcttctggttacacctttaccgactttgaaatgcactgggtgcgacaggcccctggacaagggcttgagtggatgggagatattgatcctggaactggtgatactgcctacaatctgaagttcaagggcagagtcaccatgaccacagacacatccacgagcacagcctacatggagctgaggagcctgaggtctgacgacacggccgtgtattactgtgcgttgggggcctttgtttactggggccagggaaccctggtcaccgtctcctcaggcagtactagcggtggtggctccgggggcggttccggtgggggcggcagcagcgatgttgtgatgactcagtctccactctccctgcccgtcacccctggagagccggcctccatctcctgcaggtctagtcagagtcttgcaaacagttatgggaacacctatttgtcttggtacctgcagaagccagggcagtctccacagctcctgatctatgggatttccaacagattttctggggtccctgacaggttcagtggcagtggatcaggcacagattttacactgaaaatcagcagagtggaggctgaggacgttggggtttattactgcttacaaggtacacatcagccgtacacgtttggccaggggaccaagctggagatcaaa

SEQ ID NO: 3 - protein, 466 aa, Artificial Sequence
  This sequence is synthesized in lab.
QVQLVQSGAEVKKPGASVKVSCKASGYTFTDFEMHWVRQAPGQGLEWMGDIDPGTGDTAYNLKFKGRVTMTTDTSTSTAYMELRSLRSDDTAVYYCALGAFVYWGQGTLVTVSSGSTSGGGSGGGSGGGGSSDVVMTQSPLSLPVTPGEPASISCRSSQSLANSYGNTYLSWYLQKPGQSPQLLIYGISNRFSGVPDRFSGSGSGTDFTLKISRVEAEDVGVYYCLQGTHQPYTFGQGTKLEIKTTTPAPRPPTPAPTIASQPLSLRPEACRPAAGGAVHTRGLDFACDIYIWAPLAGTCGVLLLSLVITLYCRSKRSRLLHSDYMNMTPRRPGPTRKHYQPYAPPRDFAAYRSRVKFSRSADAPAYKQGQNQLYNELNLGRREEYDVLDKRRGRDPEMGGKPRRKNPQEGLYNELQKDKMAEAYSEIGMKGERRRGKGHDGLYQGLSTATKDTYDALHMQALPPR

SEQ ID NO: 4 - protein, 561 aa, Artificial Sequence
  This sequence is synthesized in lab.
QVQLVQSGAEVKKPGASVKVSCKASGYTFTDFEMHWVRQAPGQGLEWMGDIDPGTGDTAYNLKFKGRVTMTTDTSTSTAYMELRSLRSDDTAVYYCALGAFVYWGQGTLVTVSSGSTSGGGSGGGSGGGGSSDVVMTQSPLSLPVTPGEPASISCRSSQSLANSYGNTYLSWYLQKPGQSPQLLIYGISNRFSGVPDRFSGSGSGTDFTLKISRVEAEDVGVYYCLQGTHQPYTFGQGTKLEIKTTTPAPRPPTPAPTIASQPLSLRPEACRPAAGGAVHTRGLDFACDIYIWAPLAGTCGVLLLSLVITLYCRSKRSRLLHSDYMNMTPRRPGPTRKHYQPYAPPRDFAAYRSKKRIKPIVWPSLPDHKKTLEHLCKKPRKNLNVSFNPESFLDCQIHRVDDIQARDEVEGFLQDTFPQQLEESEKQRLLGSNQEEAYVTMSSFYQNQRVKFSRSADAPAYKQGQNQLYNELNLGRREEYDVLDKRRGRDPEMGGKPRRKNPQEGLYNELQKDKMAEAYSEIGMKGERRRGKGHDGLYQGLSTATKDTYDALHMQALPPR

SEQ ID NO: 5 - protein, 737 aa, Artificial Sequence
  This sequence is synthesized in lab.
QVQLVQSGAEVKKPGASVKVSCKASGYTFTDFEMHWVRQAPGQGLEWMGDIDPGTGDTAYNLKFKGRVTMTTDTSTSTAYMELRSLRSDDTAVYYCALGAFVYWGQGTLVTVSSGSTSGGGSGGGSGGGGSSDVVMTQSPLSLPVTPGEPASISCRSSQSLANSYGNTYLSWYLQKPGQSPQLLIYGISNRFSGVPDRFSGSGSGTDFTLKISRVEAEDVGVYYCLQGTHQPYTFGQGTKLEIKTTTPAPRPPTPAPTIASQPLSLRPEACRPAAGGAVHTRGLDFACDIYIWAPLAGTCGVLLLSLVITLYCRSKRSRLLHSDYMNMTPRRPGPTRKHYQPYAPPRDFAAYRSRVKFSRSADAPAYKQGQNQLYNELNLGRREEYDVLDKRRGRDPEMGGKPRRKNPQEGLYNELQKDKMAEAYSEIGMKGERRRGKGHDGLYQGLSTATKDTYDALHMQALPPREGRGSLLTCGDVEENPGPMTNKCLLQIALLLCFSTTALSQVQLQQSGPGLVKPSHTLSLTCTVSGGSISSGGYYWSWTRQHPGMGLEWIGYISYSGSIYYTPSLKSRLTISVDTSKNQFSLKLSSVTAADTAVYYCASLDSWGSNRDYWGQGTLVTVSSGGGGSEIVLTQSPATLSLSPGERATLSCRASQSVSSYLAWYQQKPGQAPRLLIYDASNRATGIPARFSGSGSGTDFTLTISSLEPEDFAVYYCQQRSNWPLTFGGGTKVEIK

SEQ ID NO: 6 - protein, 832 aa, Artificial Sequence
  This sequence is synthesized in lab.
QVQLVQSGAEVKKPGASVKVSCKASGYTFTDFEMHWVRQAPGQGLEWMGDIDPGTGDTAYNLKFKGRVTMTTDTSTSTAYMELRSLRSDDTAVYYCALGAFVYWGQGTLVTVSSGSTSGGGSGGGSGGGGSSDVVMTQSPLSLPVTPGEPASISCRSSQSLANSYGNTYLSWYLQKPGQSPQLLIYGISNRFSGVPDRFSGSGSGTDFTLKISRVEAEDVGVYYCLQGTHQPYTFGQGTKLEIKTTTPAPRPPTPAPTIASQPLSLRPEACRPAAGGAVHTRGLDFACDIYIWAPLAGTCGVLLLSLVITLYCRSKRSRLLHSDYMNMTPRRPGPTRKHYQPYAPPRDFAAYRSKKRIKPIVWPSLPDHKKTLEHLCKKPRKNLNVSFNPESFLDCQIHRVDDIQARDEVEGFLQDTFPQQLEESEKQRLLGSNQEEAYVTMSSFYQNQRVKFSRSADAPAYKQGQNQLYNELNLGRREEYDVLDKRRGRDPEMGGKPRRKNPQEGLYNELQKDKMAEAYSEIGMKGERRRGKGHDGLYQGLSTATKDTYDALHMQALPPREGRGSLLTCGDVEENPGPMTNKCLLQIALLLCFSTTALSQVQLQQSGPGLVKPSHTLSLTCTVSGGSISSGGYYWSWTRQHPGMGLEWIGYISYSGSIYYTPSLKSRLTISVDTSKNQFSLKLSSVTAADTAVYYCASLDSWGSNRDYWGQGTLVTVSSGGGGSEIVLTQSPATLSLSPGERATLSCRASQSVSSYLAWYQQKPGQAPRLLIYDASNRATGIPARFSGSGSGTDFTLTISSLEPEDFAVYYCQQRSNWPLTFGGGTKVEIK

SEQ ID NO: 7 - DNA, 1398 bp, Artificial Sequence
  This sequence is synthesized in lab.
caggttcagctggtgcagtctggagctgaggtgaagaagcctggggcctcagtgaaggtctcctgcaaggcttctggttacacctttaccgactttgaaatgcactgggtgcgacaggcccctggacaagggcttgagtggatgggagatattgatcctggaactggtgatactgcctacaatctgaagttcaagggcagagtcaccatgaccacagacacatccacgagcacagcctacatggagctgaggagcctgaggtctgacgacacggccgtgtattactgtgcgttgggggcctttgtttactggggccagggaaccctggtcaccgtctcctcaggcagtactagcggtggtggctccgggggcggttccggtgggggcggcagcagcgatgttgtgatgactcagtctccactctccctgcccgtcacccctggagagccggcctccatctcctgcaggtctagtcagagtcttgcaaacagttatgggaacacctatttgtcttggtacctgcagaagccagggcagtctccacagctcctgatctatgggatttccaacagattttctggggtccctgacaggttcagtggcagtggatcaggcacagattttacactgaaaatcagcagagtggaggctgaggacgttggggtttattactgcttacaaggtacacatcagccgtacacgtttggccaggggaccaagctggagatcaaaaccactaccccagcaccgaggccacccaccccggctcctaccatcgcctcccagcctctgtccctgcgtccggaggcatgtagacccgcagctggtggggccgtgcatacccggggtcttgacttcgcctgcgatatctacatttgggcccctctggctggtacttgcggggtcctgctgctttcactcgtgatcactctttactgtaggagtaagaggagcaggctcctgcacagtgactacatgaacatgactccccgccgccccgggcccacccgcaagcattaccagccctatgccccaccacgcgacttcgcagcctatcgctcccgcgtgaaattcagccgcagcgcagatgctccagcctacaagcaggggcagaaccagctctacaacgaactcaatcttggtcggagagaggagtacgacgtgctggacaagcggagaggacgggacccagaaatgggcgggaagccgcgcagaaagaatccccaagagggcctgtacaacgagctccaaaaggataagatggcagaagcctatagcgagattggtatgaaaggggaacgcagaagaggcaaaggccacgacggactgtaccagggactcagcaccgccaccaaggacacctatgacgctcttcacatgcaggccctgccgcctcgg

SEQ ID NO: 8 - DNA, 1683 bp, Artificial Sequence
  This sequence is synthesized in lab.
caggttcagctggtgcagtctggagctgaggtgaagaagcctggggcctcagtgaaggtctcctgcaaggcttctggttacacctttaccgactttgaaatgcactgggtgcgacaggcccctggacaagggcttgagtggatgggagatattgatcctggaactggtgatactgcctacaatctgaagttcaagggcagagtcaccatgaccacagacacatccacgagcacagcctacatggagctgaggagcctgaggtctgacgacacggccgtgtattactgtgcgttgggggcctttgtttactggggccagggaaccctggtcaccgtctcctcaggcagtactagcggtggtggctccgggggcggttccggtgggggcggcagcagcgatgttgtgatgactcagtctccactctccctgcccgtcacccctggagagccggcctccatctcctgcaggtctagtcagagtcttgcaaacagttatgggaacacctatttgtcttggtacctgcagaagccagggcagtctccacagctcctgatctatgggatttccaacagattttctggggtccctgacaggttcagtggcagtggatcaggcacagattttacactgaaaatcagcagagtggaggctgaggacgttggggtttattactgcttacaaggtacacatcagccgtacacgtttggccaggggaccaagctggagatcaaaaccactaccccagcaccgaggccacccaccccggctcctaccatcgcctcccagcctctgtccctgcgtccggaggcatgtagacccgcagctggtggggccgtgcatacccggggtcttgacttcgcctgcgatatctacatttgggcccctctggctggtacttgcggggtcctgctgctttcactcgtgatcactctttactgtaggagtaagaggagcaggctcctgcacagtgactacatgaacatgactccccgccgccccgggcccacccgcaagcattaccagccctatgccccaccacgcgacttcgcagcctatcgctccaaaaaaaggattaagcctatcgtatggcccagtctccccgatcacaagaagactctggaacacctttgtaagaaaccaagaaaaaatttaaatgtgagtttcaatcctgaaagtttcctggactgccagattcatagggtggatgacattcaagctagagatgaagtggaaggttttctgcaagatacgtttcctcagcaactagaagaatctgagaagcagaggcttctgggatcaaatcaagaagaagcatatgtcaccatgtccagcttctaccaaaaccagcgcgtgaaattcagccgcagcgcagatgctccagcctacaagcaggggcagaaccagctctacaacgaactcaatcttggtcggagagaggagtacgacgtgctggacaagcggagaggacgggacccagaaatgggcgggaagccgcgcagaaagaatccccaagagggcctgtacaacgagctccaaaaggataagatggcagaagcctatagcgagattggtatgaaaggggaacgcagaagaggcaaaggccacgacggactgtaccagggactcagcaccgccaccaaggacacctatgacgctcttcacatgcaggccctgccgcctcgg

SEQ ID NO: 9 - DNA, 2211 bp, Artificial Sequence
  This sequence is synthesized in lab.
caggttcagctggtgcagtctggagctgaggtgaagaagcctggggcctcagtgaaggtctcctgcaaggcttctggttacacctttaccgactttgaaatgcactgggtgcgacaggcccctggacaagggcttgagtggatgggagatattgatcctggaactggtgatactgcctacaatctgaagttcaagggcagagtcaccatgaccacagacacatccacgagcacagcctacatggagctgaggagcctgaggtctgacgacacggccgtgtattactgtgcgttgggggcctttgtttactggggccagggaaccctggtcaccgtctcctcaggcagtactagcggtggtggctccgggggcggttccggtgggggcggcagcagcgatgttgtgatgactcagtctccactctccctgcccgtcacccctggagagccggcctccatctcctgcaggtctagtcagagtcttgcaaacagttatgggaacacctatttgtcttggtacctgcagaagccagggcagtctccacagctcctgatctatgggatttccaacagattttctggggtccctgacaggttcagtggcagtggatcaggcacagattttacactgaaaatcagcagagtggaggctgaggacgttggggtttattactgcttacaaggtacacatcagccgtacacgtttggccaggggaccaagctggagatcaaaaccactaccccagcaccgaggccacccaccccggctcctaccatcgcctcccagcctctgtccctgcgtccggaggcatgtagacccgcagctggtggggccgtgcatacccggggtcttgacttcgcctgcgatatctacatttgggcccctctggctggtacttgcggggtcctgctgctttcactcgtgatcactctttactgtaggagtaagaggagcaggctcctgcacagtgactacatgaacatgactccccgccgccccgggcccacccgcaagcattaccagccctatgccccaccacgcgacttcgcagcctatcgctcccgcgtgaaattcagccgcagcgcagatgctccagcctacaagcaggggcagaaccagctctacaacgaactcaatcttggtcggagagaggagtacgacgtgctggacaagcggagaggacgggacccagaaatgggcgggaagccgcgcagaaagaatccccaagagggcctgtacaacgagctccaaaaggataagatggcagaagcctatagcgagattggtatgaaaggggaacgcagaagaggcaaaggccacgacggactgtaccagggactcagcaccgccaccaaggacacctatgacgctcttcacatgcaggccctgccgcctcgggagggaaggggttctctcctgacctgcggcgatgtggaggagaaccccggacccatgaccaacaagtgtctcctccaaattgctctcctgttgtgcttctccactacagctctttcccaggtgcagctacagcagtcgggcccaggactggtgaagccttcacacaccctgtccctcacctgcactgtctctggtggctccatcagcagtggtggttactactggagttggacccgtcagcacccagggatgggcctggagtggattggatacatctcttacagtgggagtatctattacactccgtccctcaagagtcgacttaccatatcagtggacacgtctaagaaccagttctccctgaagctgagctctgtgactgccgcggacacggccgtatattactgtgcgagtttggattcctggggatctaaccgtgactactggggccagggaaccctggtcaccgtctcgagtggaggtggtggatccgaaattgtgttgacgcagtctccagccaccctgtctttgtctccaggggaaagagccaccctctcctgcagggccagtcagagtgttagcagctacttagcctggtaccaacagaaacctggccaggctcccaggctcctcatctatgatgcatccaacagggccactggcatcccagccaggttcagtggcagtgggtctgggacagacttcactctcaccatcagcagcctagagcctgaagattttgcagtttattactgtcagcagcgtagcaactggccgctcactttcggcggagggaccaaggtggagattaag

SEQ ID NO: 10 - DNA, 2534 bp, Artificial Sequence
  This sequence is synthesized in lab.
caggttcagctggtgcagtctggagctgaggtgaagaagcctggggcctcagtgaaggtctcctgcaaggcttctggttacacctttaccgactttgaaatgcactgggtgcgacaggcccctggacaagggcttgagtggatgggagatattgatcctggaactggtgatactgcctacaatctgaagttcaagggcagagtcaccatgaccacagacacatccacgagcacagcctacatggagctgaggagcctgaggtctgacgacacggccgtgtattactgtgcgttgggggcctttgtttactggggccagggaaccctggtcaccgtctcctcaggcagtactagcggtggtggctccgggggcggttccggtgggggcggcagcagcgatgttgtgatgactcagtctccactctccctgcccgtcacccctggagagccggcctccatctcctgcaggtctagtcagagtcttgcaaacagttatgggaacacctatttgtcttggtacctgcagaagccagggcagtctccacagctcctgatctatgggatttccaacagattttctggggtccctgacaggttcagtggcagtggatcaggcacagattttacactgaaaatcagcagagtggaggctgaggacgttggggtttattactgcttacaaggtacacatcagccgtacacgtttggccaggggaccaagctggagatcaaaaccactaccccagcaccgaggccacccaccccggctcctaccatcgcctcccagcctctgtccctgcgtccggaggcatgtagacccgcagctggtggggccgtgcatacccggggtcttgacttcgcctgcgatatctacatttgggcccctctggctggtacttgcggggtcctgctgctttcactcgtgatcactctttactgtaggagtaagaggagcaggctcctgcacagtgactacatgaacatgactccccgccgccccgggcccacccgcaagcattaccagccctatgccccaccacgcgacttcgcagcctatcgctccaaaaaaaggattaagcctatcgtatggcccagtctccccgatcacaagaagactctggaacacctttgtaagaaaccaagaaaaaatttaaatgtgagtttcaatcctgaaagtttcctggactgccagattcatagggtggatgacattcaagctagagatgaagtggaaggttttctgcaagatacgtttcctcagcaactagaagaatctgagaagcagaggcttctgggatcaaatcaagaagaagcatatgtcaccatgtccagcttctaccaaaaccagcgcgtgaaattcagccgcagcgcagatgctccagcctacaagcaggggcagaaccagctctacaacgaactcaatcttggtcggagagaggagtacgacgtgctggacaagcggagaggacgggacccagaaatgggcgggaagccgcgcagaaagaatccccaagagggcctgtacaacgagctccaaaaggataagatggcagaagcctatagcgagattggtatgaaaggggaacgcagaagaggcaaaggccacgacggactgtaccagggactcagcaccgccaccaaggacacctatgacgctcttcacatgcaggccctgccgcctcgggagggaaggggttctctcctgacctgcggcgatgtggaggagaaccccggacccatgaccaacaagtgtctcctccaaattgctctcctgttgtgcttctccactacagctctttcccaggtgcagctacagcagtcgggcccaggactggtgaagccttcacacaccctgtccctcacctgcactgtctctggtggctccatcagcagtggtggttactactggagttggacccgtcagcacccagggatgggcctggagtggattggatacatctcttacagtgggagtatctattacactccgtccctcaagagtcgacttaccatatcagtggacacgtctaagaaccagttctccctgaagctgagctctgtgactgccgcggacacggccgtatattactgtgcgagtttggattcctggggatctaaccgtgactactggggccagggaaccctggtcaccgtctcgagtggaggtggtggatccgaaattgtgttgacgcagtctccagccaccctgtctttgtctccaggggaaagagccaccctctcctgcagggccagtcagagtgttagcagctacttagcctggtaccaacagaaacctggccaggctcccaggctcctcatctatgatgcatccaacagggccactggcatcccagccaggttcagtggcagtgggtctgggacagacttcactctcaccatcagcagcctagagcctgaagattttgcagtttattactgtcagcagcgtagcaactggccgctcactttcggcggagggaccaaggtggagattaagcgctcactttcggcggagggaccaaggtggagattaag